European Patent Application EP 4 137 148 A1, published February 22, 2023. Title: POPULATIONS OF SMALL EXTRACELLULAR VESICLES FOR USE IN THE TREATMENT OF OBESITY. Applicant: UNIVERSIDADE DE SANTIAGO DE COMPOSTELA Centre National de la Recherche Scientifique (CNRS) INSTITUT NATIONAL DE LA SANTÉ ET DE LA RECHERCHE MÉDICALE (INSERM) Université d'Angers. The sequence listing filed with the application follows.

SEQUENCE LISTING (38 sequences)

SEQ ID NO: 1 - protein, 560 aa, Artificial Sequence
  AMPKα1-DN mutant protein amino acid sequence
MEQKLISEEDLGGGEKQKHDGRVKIGHYILGDTLGVGTFGKVKVGKHELTGHKVAVKILNRQKIRSLDVVGKIRREIQNLKLFRHPHIIKLYQVISTPSDIFMVMEYVSGGELFDYICKNGRLDEKESRRLFQQILSGVDYCHRHMVVHRDLKPENVLLDAHMNAKIAAFGLSNMMSDGEFLRTSCGSPNYAAPEVISGRLYAGPEVDIWSSGVILYALLCGTLPFDDDHVPTLFKKICDGIFYTPQYLNPSVISLLKHMLQVDPMKRATIKDIREHEWFKQDLPKYLFPEDPSYSSTMIDDEALKEVCEKFECSEEEVLSCLYNRNHQDPLAVAYHLIIDNRRIMNEAKDFYLATSPPDSFLDDHHLTRPHPERVPFLVAETPRARHTLDELNPQKSKHQGVRKAKWHLGIRSQSRPNDIMAEVCRAIKQLDYEWKVVNPYYLRVRRKNPVTSTFSKMSLQLYQVDSRTYLLDFRSIDDEITEAKSGTATPQRSGSISNYRSCQRSDSDAEAQGKPSEVSLTSSVTSLDSSPVDVAPRPGSHTIEFFEMCANLIKILAQ

SEQ ID NO: 2 - protein, 1683 aa, Artificial Sequence
  Polynucleotide sequence encoding for the dominant negative AMP-activated protein kinase alpha 1 (AMPKα1) mutant protein.
ATGGAGCAGAAGCTTATCTCCGAGGAGGACCTCGGTGGCGGCGAGAAGCAGAAGCACGACGGGCGGGTGAAGATCGGCCACTACATCCTGGGGGACACGCTGGGCGTCGGCACCTTCGGGAAAGTGAAGGTGGGCAAGCACGAGTTGACTGGACATAAAGTTGCTGTGAAGATACTCAACCGGCAGAAGATTCGAAGCCTGGACGTGGTCGGGAAAATCCGCAGAGAGATCCAGAACCTGAAGCTTTTCAGGCACCCTCATATAATCAAACTGTACCAGGTCATCAGTACACCGTCTGATATTTTCATGGTCATGGAATATGTCTCAGGAGGAGAGCTATTTGATTATATCTGTAAAAATGGAAGGTTGGACGAAAAGGAGAGTCGACGTCTGTTCCAGCAGATCCTTTCTGGTGTGGACTATTGTCACAGGCATATGGTGGTCCACAGAGATTTGAAACCTGAAAACGTCCTGCTTGATGCACACATGAATGCAAAGATAGCCGCCTTCGGTCTTTCAAACATGATGTCAGATGGTGAATTTTTAAGAACGAGCTGTGGCTCGCCCAATTATGCTGCACCAGAAGTAATTTCAGGAAGATTGTACGCAGGCCCTGAAGTAGACATCTGGAGCAGCGGGGTCATTCTCTATGCTTTGCTGTGTGGAACTCTCCCTTTTGATGATGACCACGTGCCAACTCTTTTTAAGAAGATATGTGACGGGATATTTTATACCCCTCAGTATTTGAATCCCTCTGTAATAAGCCTTTTGAAGCATATGCTGCAGGTAGATCCTATGAAGAGGGCCACAATAAAAGATATCAGGGAACATGAATGGTTTAAGCAGGACCTTCCAAAATATCTCTTTCCTGAAGACCCGTCTTATAGTTCAACCATGATTGATGATGAAGCCTTAAAAGAAGTGTGTGAGAAGTTCGAGTGCTCAGAGGAGGAGGTCCTCAGCTGCCTGTACAACAGAAACCACCAGGACCCACTGGCAGTTGCCTACCACCTCATAATAGACAACAGGAGAATAATGAACGAAGCCAAAGATTTCTACTTGGCAACAAGCCCACCCGATTCTTTCCTCGATGATCACCATTTAACTCGGCCTCACCCTGAGAGAGTACCATTCTTGGTTGCCGAAACACCAAGGGCCCGACACACCCTAGATGAATTAAACCCACAGAAATCCAAACACCAAGGCGTACGGAAGGCAAAGTGGCATTTGGGGATTCGAAGTCAAAGCCGACCCAATGACATCATGGCAGAAGTGTGTAGAGCAATCAAGCAGTTGGACTATGAATGGAAGGTTGTAAACCCCTATTATTTGCGTGTGCGAAGGAAGAACCCTGTGACAAGCACATTTTCCAAAATGAGTCTACAGCTATACCAAGTGGATAGTAGGACTTACTTATTGGATTTCCGAAGTATTGATGATGAGATTACAGAAGCCAAATCAGGGACTGCTACTCCACAGAGATCGGGATCCATCAGCAACTATCGATCTTGCCAAAGGAGCGACTCCGACGCCGAGGCTCAAGGAAAGCCCTCAGAAGTCTCTCTTACCTCATCCGTGACCTCCCTCGACTCCTCTCCTGTTGACGTAGCTCCAAGACCAGGAAGTCACACGATAGAATTTTTTGAAATGTGTGCAAATCTAATTAAAATTCTTGCACAGTAA

SEQ ID NO: 3 - DNA, 741 bp, Artificial Sequence
  Steroidogenic factor 1 (SF1) polynucleotide sequence.
aaaacaaaacaaaacaaaacaaaacaaaacaaaacaaacaaacaaacaaacaaacaaaaacccttctttcctacctggtcctagtacccacatagtcctacctgaagtccctgaagccacacccttagcccagcagtcttggcacaacctcagtttccccagctaccaatggaccatatctgcagctcccagagaagccaccaaaaaggccacacaaaccccacctgatgggttccaccatgccatttctccacactagccattctgactcctcactcagatctgggacaagctggaccacgcagcccaggcaaggacccagggaggaagccattcaaggggagaaactcccagcctggtaagggagcaggccataaatcaggtcccactcccacccagtcgctaacaagccgctgcctatctgcctacatggggtccctgcctcaggctccctcatcagcctggacagccagctggccaaggtctctccagtgccttggcctctgcccccacccagggcccccataaagatagggatatttttttttcttttagaagagtgaaaaaagatatagacccaaatgaagagaaacaccaacaaaggaggagaaaggcctgcagagtcacgtgggggcagagaccaattgggcctccggtggcccccccacccacgaggggaggaggaaaggacgatcggacagggccagtttccagtccgccgctgcccgcccgctgctgggt

SEQ ID NO: 4 - DNA, 2476 bp, Artificial Sequence
  Polyucleotide sequence encoding a AMPKα1-DN mutant protein operably linked and under the control of the SF1 promoter.
aaaacaaaacaaaacaaaacaaaacaaaacaaaacaaacaaacaaacaaacaaacaaaaacccttctttcctacctggtcctagtacccacatagtcctacctgaagtccctgaagccacacccttagcccagcagtcttggcacaacctcagtttccccagctaccaatggaccatatctgcagctcccagagaagccaccaaaaaggccacacaaaccccacctgatgggttccaccatgccatttctccacactagccattctgactcctcactcagatctgggacaagctggaccacgcagcccaggcaaggacccagggaggaagccattcaaggggagaaactcccagcctggtaagggagcaggccataaatcaggtcccactcccacccagtcgctaacaagccgctgcctatctgcctacatggggtccctgcctcaggctccctcatcagcctggacagccagctggccaaggtctctccagtgccttggcctctgcccccacccagggcccccataaagatagggatatttttttttcttttagaagagtgaaaaaagatatagacccaaatgaagagaaacaccaacaaaggaggagaaaggcctgcagagtcacgtgggggcagagaccaattgggcctccggtggcccccccacccacgaggggaggaggaaaggacgatcggacagggccagtttccagtccgccgctgcccgcccgctgctgggtaccgtttaaactcgaggtcgacggtatcgataagcttgatatcgaattcgccatggagcagaagcttatctccgaggaggacctcggtggcggcgagaagcagaagcacgacgggcgggtgaagatcggccactacatcctgggggacacgctgggcgtcggcaccttcgggaaagtgaaggtgggcaagcacgagttgactggacataaagttgctgtgaagatactcaaccggcagaagattcgaagcctggacgtggtcgggaaaatccgcagagagatccagaacctgaagcttttcaggcaccctcatataatcaaactgtaccaggtcatcagtacaccgtctgatattttcatggtcatggaatatgtctcaggaggagagctatttgattatatctgtaaaaatggaaggttggacgaaaaggagagtcgacgtctgttccagcagatcctttctggtgtggactattgtcacaggcatatggtggtccacagagatttgaaacctgaaaacgtcctgcttgatgcacacatgaatgcaaagatagccgccttcggtctttcaaacatgatgtcagatggtgaatttttaagaacgagctgtggctcgcccaattatgctgcaccagaagtaatttcaggaagattgtacgcaggccctgaagtagacatctggagcagcggggtcattctctatgctttgctgtgtggaactctcccttttgatgatgaccacgtgccaactctttttaagaagatatgtgacgggatattttatacccctcagtatttgaatccctctgtaataagccttttgaagcatatgctgcaggtagatcctatgaagagggccacaataaaagatatcagggaacatgaatggtttaagcaggaccttccaaaatatctctttcctgaagacccgtcttatagttcaaccatgattgatgatgaagccttaaaagaagtgtgtgagaagttcgagtgctcagaggaggaggtcctcagctgcctgtacaacagaaaccaccaggacccactggcagttgcctaccacctcataatagacaacaggagaataatgaacgaagccaaagatttctacttggcaacaagcccacccgattctttcctcgatgatcaccatttaactcggcctcaccctgagagagtaccattcttggttgccgaaacaccaagggcccgacacaccctagatgaattaaacccacagaaatccaaacaccaaggcgtacggaaggcaaagtggcatttggggattcgaagtcaaagccgacccaatgacatcatggcagaagtgtgtagagcaatcaagcagttggactatgaatggaaggttgtaaacccctattatttgcgtgtgcgaaggaagaaccctgtgacaagcacattttccaaaatgagtctacagctataccaagtggatagtaggacttacttattggatttccgaagtattgatgatgagattacagaagccaaatcagggactgctactccacagagatcgggatccatcagcaactatcgatcttgccaaaggagcgactccgacgccgaggctcaaggaaagccctcagaagtctctcttacctcatccgtgacctccctcgactcctctcctgttgacgtagctccaagaccaggaagtcacacgatagaattttttgaaatgtgtgcaaatctaattaaaattcttgcacagtaa

SEQ ID NO: 5 - protein, 449 aa, Artificial Sequence
  Fusion protein: Neurotrophic rabies virus (RVG) peptide fused to lysosome-associated membrane protein 2b (Lamp2b).
MCLSPVKGAKLILIFLFLGAVQSNALIVNLTDSKGTCLYARYTIWMPENPRPGTPCDIFTNSRGKRASNGSGGAEWEMNFTITYETTNQTNKTITIAVPDKATHDGSSCGDDRNSAKIMIQFGFAVSWAVNFTKEASHYSIHDIVLSYNTSDSTVFPGAVAKGVHTVKNPENFKVPLDVIFKCNSVLTYNLTPVVQKYWGIHLQAFVQNGTVSKNEQVCEEDQTPTTVAPIIHTTAPSTTTTLTPTSTPTPTPTPTPTVGNYSIRNGNTTCLLATMGLQLNITEEKVPFIFNINPATTNFTGSCQPQSAQLRLNNSQIKYLDFIFAVKNEKRFYLKEVNVYMYLANGSAFNISNKNLSFWDAPLGSSYMCNKEQVLSVSRAFQINTFNLKVQPFNVTKGQYSTAQECSLDDDTILIPIIVGAGLSGLIIVIVIAYLIGRRKTYAGYQTL

SEQ ID NO: 6 - DNA, 92 bp, Artificial Sequence
  RVG primers -F
tcgatacaccatttggatgcccgagaatccgagaccagggacaccttgtgacatttttaccaatagcagagggaagagagcatccaacgggt

SEQ ID NO: 7 - DNA, 92 bp, Artificial Sequence
  RVG primer - R
ccggacccgttggatgctctcttccctctgctattggtaaaaatgtcacaaggtgtccctggtctcggattctcgggcatccaaatggtgta

SEQ ID NO: 8 - DNA, 21 bp, Artificial Sequence
  AMPK primer- F
acggccgagaagcagaagcac

SEQ ID NO: 9 - DNA, 20 bp, Artificial Sequence
  AMPK primer -R
tcgtgcttgcccaccttcac

SEQ ID NO: 10 - DNA, 19 bp, Artificial Sequence
  GAPDH Primer-F
agtatgtcgtggagtctac

SEQ ID NO: 11 - DNA, 19 bp, Artificial Sequence
  GAPDH Primer-R
catacttggcaggtttctc

SEQ ID NO: 12 - DNA, 21 bp, Artificial Sequence
  STAR primer F
agttcgacgtcggagctctct

SEQ ID NO: 13 - DNA, 20 bp, Artificial Sequence
  STAR primer R
tacttagcacttcgtccccg

SEQ ID NO: 14 - DNA, 20 bp, Artificial Sequence
  P450scc primer F
gattgcggagctggagatga

SEQ ID NO: 15 - DNA, 20 bp, Artificial Sequence
  P450scc primer R
tcttttctggtcacggctgg

SEQ ID NO: 16 - DNA, 20 bp, Artificial Sequence
  17β-HSD3 primer F
ctgagcacttccggtgagag

SEQ ID NO: 17 - DNA, 20 bp, Artificial Sequence
  17β-HSD3 primer R
ggcctttcctccttgactcc

SEQ ID NO: 18 - DNA, 20 bp, Artificial Sequence
  LH β primer F
gagttctgcccagtctgcat

SEQ ID NO: 19 - DNA, 22 bp, Artificial Sequence
  LH β primer R
aggaaaggagactatggggtct

SEQ ID NO: 20 - DNA, 22 bp, Artificial Sequence
  S11 primer F
cattcagacggagcgtgcttac

SEQ ID NO: 21 - DNA, 20 bp, Artificial Sequence
  S11 primer R
tgcatcttcatcttcgtcac

SEQ ID NO: 22 - DNA, 20 bp, Artificial Sequence
  Atp2a2 primer F
tccgctacctcatctcatcc

SEQ ID NO: 23 - DNA, 19 bp, Artificial Sequence
  Atp2a2 primer R
caggtctggaggattgaac

SEQ ID NO: 24 - DNA, 21 bp, Artificial Sequence
  Gdp2 primer F
gaaggggactattcttgtggg

SEQ ID NO: 25 - DNA, 21 bp, Artificial Sequence
  Gdp2 primer R
ggatgtcaaattcgggtgtgt

SEQ ID NO: 26 - DNA, 20 bp, Artificial Sequence
  Pparγ primer F
tcgctgatgcactgcctatg

SEQ ID NO: 27 - DNA, 21 bp, Artificial Sequence
  Pparγ primer R
gagaggtccacagagctgatt

SEQ ID NO: 28 - DNA, 21 bp, Artificial Sequence
  Ryr1 primer F
cagtttttgcggacggatgat

SEQ ID NO: 29 - DNA, 20 bp, Artificial Sequence
  Ryr1 primer R
caccggcctccacagtattg

SEQ ID NO: 30 - DNA, 25 bp, Artificial Sequence
  Sln primer F
gaggtggagagactgaggtccttgg

SEQ ID NO: 31 - DNA, 21 bp, Artificial Sequence
  Sln primer R
gaagctcggggcacacagcag

SEQ ID NO: 32 - DNA, 22 bp, Artificial Sequence
  Ucp3 primer F
gagatggtgacctacgacatca

SEQ ID NO: 33 - DNA, 22 bp, Artificial Sequence
  Ucp3 primer R
gcgttcatgtatcgggtcttta

SEQ ID NO: 34 - DNA, 20 bp, Artificial Sequence
  SF1-AMPKα1-DN primer F
aaacaccaaggcgtacggaa

SEQ ID NO: 35 - DNA, 20 bp, Artificial Sequence
  SF1-AMPKα1-DN primer R
tggcggccgctctagattac

SEQ ID NO: 36 - DNA, 20 bp, Artificial Sequence
  HPRT primer F
ggttaagcagtacagcccca

SEQ ID NO: 37 - DNA, 20 bp, Artificial Sequence
  HPRT primer R
tccaacacttcgagaggtcc

SEQ ID NO: 38 - DNA, 1378 bp, Artificial Sequence
  Nucleotide sequence of the fusion protein made of the Neurotrophic rabies virus (RVG) peptide fused to lysosome-associated membrane protein 2b (Lamp2b).
gctagcggtcgccaccatgtgcctctctccggttaaaggcgcaaagctcatcctgatctttctgttcctaggagccgttcagtccaatgcattgatagttaatttgacagattcaaagggtacttgcctttatgctcgatacaccatttggatgcccgagaatccgagaccagggacaccttgtgacatttttaccaatagcagagggaagagagcatccaacgggtccggaggtgcagaatgggagatgaatttcacaataacatatgaaactacaaaccaaaccaataaaactataaccattgcagtacctgacaaggcgacacacgatggaagcagttgtggggatgaccggaatagtgccaaaataatgatacaatttggattcgctgtctcttgggctgtgaattttaccaaggaagcatctcattattcaattcatgacatcgtgctttcctacaacactagtgatagcacagtatttcctggtgctgtagctaaaggagttcatactgttaaaaatcctgagaatttcaaagttccattggatgtcatctttaagtgcaatagtgttttaacttacaacctgactcctgtcgttcagaaatattggggtattcacctgcaagcttttgtccaaaatggtacagtgagtaaaaatgaacaagtgtgtgaagaagaccaaactcccaccactgtggcacccatcattcacaccactgccccgtcgactacaactacactcactccaacttcaacacccactccaactccaactccaactccaaccgttggaaactacagcattagaaatggcaatactacctgtctgctggctaccatggggctgcagctgaacatcactgaggagaaggtgcctttcatttttaacatcaaccctgccacaaccaacttcaccggcagctgtcaacctcaaagtgctcaacttaggctgaacaacagccaaattaagtatcttgactttatctttgctgtgaaaaatgaaaaacggttctatctgaaggaagtgaatgtctacatgtatttggctaatggctcagctttcaacatttccaacaagaaccttagcttctgggatgcccctctgggaagttcttatatgtgcaacaaagagcaggtgctttctgtgtctagagcgtttcagatcaacacctttaacctaaaggtgcaaccttttaatgtgacaaaaggacagtattctacagcccaggagtgttcgctggatgatgacaccattctaataccaattatagttggtgctggtctttcaggcttgattatcgttatagtgattgcttacctaattggcagaagaaagacctatgctggatatcagactctgtaacactaaggatcc